European Patent Application EP 4 317 173 A1, published February 7, 2024. Title: PEPTIDE, AND COMPOSITION CONTAINING THE PEPTIDE AS ACTIVE INGREDIENT. Applicant: MORINAGA MILK INDUSTRY CO., LTD. KYOTO UNIVERSITY. The sequence listing filed with the application follows.

SEQUENCE LISTING (1 sequence)

SEQ ID NO: 1 - protein, 6 aa, Artificial Sequence
  Synthetic peptide, or Natural peptide
NLPPLT